European Patent Application EP 4 180 457 A1, published May 17, 2023. Title: ANTI-CLDN-18.2 ANTIBODY AND USE THEREOF. Applicant: SHANGHAI JUNSHI BIOSCIENCES CO., LTD. SUZHOU JUNMENG BIOSCIENCES CO., LTD. Application PCT/CN2021/106125. The sequence listing filed with the application follows.

SEQUENCE LISTING (101 sequences)

SEQ ID NO: 1 - protein, 5 aa, Artificial Sequence
NFGMH

SEQ ID NO: 2 - protein, 17 aa, Artificial Sequence
CISSGSGTIYYADTVKG

SEQ ID NO: 3 - protein, 9 aa, Artificial Sequence
AYYGNGFSF

SEQ ID NO: 4 - protein, 10 aa, Artificial Sequence
SASSIFSYIF

SEQ ID NO: 5 - protein, 7 aa, Artificial Sequence
LTSKLAS

SEQ ID NO: 6 - protein, 8 aa, Artificial Sequence
HQWKITHT

SEQ ID NO: 7 - protein, 17 aa, Artificial Sequence
KSSQSLLNSGNQKNYLT

SEQ ID NO: 8 - protein, 7 aa, Artificial Sequence
WASTRES

SEQ ID NO: 9 - protein, 9 aa, Artificial Sequence
QNVYSYPLT

SEQ ID NO: 10 - protein, 5 aa, Artificial Sequence
NYGMN

SEQ ID NO: 11 - protein, 17 aa, Artificial Sequence
WINTYTGESTYADDFKG

SEQ ID NO: 12 - protein, 10 aa, Artificial Sequence
TLGYGNSLAY

SEQ ID NO: 13 - protein, 17 aa, Artificial Sequence
KSSQSLLNSGNQRNYLT

SEQ ID NO: 14 - protein, 7 aa, Artificial Sequence
WASTRES

SEQ ID NO: 15 - protein, 9 aa, Artificial Sequence
QNNYFYPFT

SEQ ID NO: 16 - protein, 5 aa, Artificial Sequence
SFGVS

SEQ ID NO: 17 - protein, 16 aa, Artificial Sequence
AIWAGGNRNYNSALMS

SEQ ID NO: 18 - protein, 9 aa, Artificial Sequence
GSYGSSFAN

SEQ ID NO: 19 - protein, 17 aa, Artificial Sequence
KSSQSLLNSGNQKNYLT

SEQ ID NO: 20 - protein, 7 aa, Artificial Sequence
WASTRDS

SEQ ID NO: 21 - protein, 9 aa, Artificial Sequence
QNAYFYPFT

SEQ ID NO: 22 - protein, 5 aa, Artificial Sequence
NYGMN

SEQ ID NO: 23 - protein, 17 aa, Artificial Sequence
WINTYTGESTYADDFKG

SEQ ID NO: 24 - protein, 9 aa, Artificial Sequence
SYNGNSLPY

SEQ ID NO: 25 - protein, 17 aa, Artificial Sequence
KSSQSLLNSGNQKNYLT

SEQ ID NO: 26 - protein, 7 aa, Artificial Sequence
WASTRES

SEQ ID NO: 27 - protein, 9 aa, Artificial Sequence
QNDYSYPLT

SEQ ID NO: 28 - protein, 5 aa, Artificial Sequence
SYGMS

SEQ ID NO: 29 - protein, 17 aa, Artificial Sequence
TISGGDSYTYYPDSVRG

SEQ ID NO: 30 - protein, 9 aa, Artificial Sequence
SYNGNSLPY

SEQ ID NO: 31 - protein, 17 aa, Artificial Sequence
KSSQSLLNSGNQKNYLT

SEQ ID NO: 32 - protein, 7 aa, Artificial Sequence
WASTRES

SEQ ID NO: 33 - protein, 9 aa, Artificial Sequence
QNTYSFPLT

SEQ ID NO: 34 - protein, 5 aa, Artificial Sequence
NYGMN

SEQ ID NO: 35 - protein, 17 aa, Artificial Sequence
WINTYTGEPTYADDFKG

SEQ ID NO: 36 - protein, 2 aa, Artificial Sequence
GY

SEQ ID NO: 37 - protein, 5 aa, Artificial Sequence
NYLIE

SEQ ID NO: 38 - protein, 17 aa, Artificial Sequence
VINPGSGGTNYNEKFKG

SEQ ID NO: 39 - protein, 11 aa, Artificial Sequence
PHDGYYFWFAY

SEQ ID NO: 40 - protein, 17 aa, Artificial Sequence
WINTYTGESTYADGFTG

SEQ ID NO: 41 - protein, 17 aa, Artificial Sequence
SISSGSGTIYYADSVKG

SEQ ID NO: 42 - protein, 118 aa, Artificial Sequence
DVQLVESGGGLVQPGGSRKLSCAASGFTLNNFGMHWVRQAPEKGLEWVACISSGSGTIYYADTVKGRFTISRDNPKNTLFLQMTSLRSEDTAMYYCARAYYGNGFSFWGQGTLVTVSS

SEQ ID NO: 43 - protein, 105 aa, Artificial Sequence
QIVLTQSPTLMSASPGEKVTMTCSASSIFSYIFWSQQKPRSSPKPWIYLTSKLASGVPVRFSGSGSGTSYSLTISTMEAEDAATYYCHQWKITHTFGAGTKLELK

SEQ ID NO: 44 - protein, 113 aa, Artificial Sequence
DIVMTQSPSSLTVTAGEKVTMSCKSSQSLLNSGNQKNYLTWYQQKPGQPPKLLIYWASTRESGVPDRFTGSGSGTDFTLTISSVQAEDLAIYYCQNVYSYPLTFGAGTKLEIK

SEQ ID NO: 45 - protein, 118 aa, Artificial Sequence
QIQLVQSGPELKKPGETVKISCKASGYTFTNYGMNWVKQAPGKGLKWMGWINTYTGESTYADDFKGRFAFSSETSARTAYLQINNLKNEDMATYFCATLGYGNSLAYWGQGTLVTVSS

SEQ ID NO: 46 - protein, 113 aa, Artificial Sequence
DIVMTQYPSFLTVTTGEKVTMSCKSSQSLLNSGNQRNYLTWYQQKPGQPPKLLIYWASTRESGVPDRFAGSGSGTDFTLTISSVQAEDLAIYYCQNNYFYPFTFGSGTKLEVK

SEQ ID NO: 47 - protein, 117 aa, Artificial Sequence
QVQLKESGPGLVAPSQSLSITCTVSGFSLTSFGVSWVRQPPGKGLEWLGAIWAGGNRNYNSALMSRLSISKDNSKSQVFLKMTSLQTDDTAIYYCARGSYGSSFANWGQGTLVTVSS

SEQ ID NO: 48 - protein, 113 aa, Artificial Sequence
DIVMTQSPSFLTVTAGEKVTMSCKSSQSLLNSGNQKNYLTWYQQKPGQPPKLLIYWASTRDSGVPDRFTGSGSGTDFTLTITSVQAEDLAVFYCQNAYFYPFTFGSGTKLEIK

SEQ ID NO: 49 - protein, 118 aa, Artificial Sequence
QIQLVQSGPELKKPGETVKISCKASGYTFTNYGMNWVKQAPGKGLKWMGWINTYTGESTYADDFKGRFAFSSETSARTAYLQINNLKNEGMATYFCARSYNGNSLPYWGQGTLVTVSS

SEQ ID NO: 50 - protein, 113 aa, Artificial Sequence
DIVMTQSPSFLTVTAGEKVTMSCKSSQSLLNSGNQKNYLTWYQQKPGQPPKLLIYWASTRESGVPDRFTGSGSGTDFTLTISSVQAEDLAVYYCQNDYSYPLTFGAGTKLELK

SEQ ID NO: 51 - protein, 118 aa, Artificial Sequence
EVKLVESGGGLVKPGGSLKLSCAASGFTFSSYGMSWVRQTPEKRLECVATISGGDSYTYYPDSVRGRFTISRDIAKNNLYLQMSSLRSEDTALYYCARSYNGNSLPYWGQGTLVTVSS

SEQ ID NO: 52 - protein, 113 aa, Artificial Sequence
DIVMTQSPSSLTVTAGEKVTMSCKSSQSLLNSGNQKNYLTWYQQKPGQPPKLLIYWASTRESGVPDRFTGSGSGIDFTLTISSVQAEDLAFYYCQNTYSFPLTFGAGTRLDLK

SEQ ID NO: 53 - protein, 111 aa, Artificial Sequence
QIQLVQSGPELKKPGETVKISCKASGYTFTNYGMNWVKQAPGKGLKWMGWINTYTGEPTYADDFKGRFAFSLETSASTAYLQINNLKNEDTATYFCARGYWGQGTTLTVSS

SEQ ID NO: 54 - protein, 120 aa, Artificial Sequence
QVQLQQSGAELVRPGTSVKVSCKASGYAFTNYLIEWVKQRPGQGLEWIGVINPGSGGTNYNEKFKGKATLTADKSSSTAYMQLSSLTSDDSAVYFCARPHDGYYFWFAYWGQGTLVTVSS

SEQ ID NO: 55 - protein, 118 aa, Artificial Sequence
QIQLVQSGSELKKPGESVKVSCKASGYTFTNYGMNWVRQAPGQGLEWMGWINTYTGESTYADGFTGRFVFSSDTSARTAYLQISSLKAEDTAVYFCATLGYGNSLAYWGQGTLVTVSS

SEQ ID NO: 56 - protein, 113 aa, Artificial Sequence
DIVMTQSPDSLAVSLGERATINCKSSQSLLNSGNQRNYLTWYQQKPGQPPKLLIYWASTRESGVPDRFSGSGSGTDFTLTISSLQAEDVAVYYCQNNYFYPFTFGQGTKLEIK

SEQ ID NO: 57 - protein, 118 aa, Artificial Sequence
QVQLVQSGSELKKPGESVKVSCKASGYTFTNYGMNWVRQAPGQGLEWMGWINTYTGESTYADGFTGRFVFSMDTSASTAYLQISSLKAEDMAMYFCATLGYGNSLAYWGQGTLVTVSS

SEQ ID NO: 58 - protein, 118 aa, Artificial Sequence
EVQLVESGGGLVKPGGSLRLSCAASGFTFSSYGMSWVRQAPGKGLEWVSTISGGDSYTYYPDSVRGRFTISRDNAKNSLYLQMNSLRAEDTAVYYCARSYNGNSLPYWGQGTLVTVSS

SEQ ID NO: 59 - protein, 118 aa, Artificial Sequence
EVQLVESGGGLVKPGGSLRLSCAASGFTFSSYGMSWVRQAPGKGLESVSTISGGDSYTYYPDSVRGRFTISRDIAKNSLYLQMNSLRAEDTAVYYCARSYNGNSLPYWGQGTLVTVSS

SEQ ID NO: 60 - protein, 118 aa, Artificial Sequence
EVQLVESGGGLVQPGGSLRLSCAASGFTLNNFGMHWVRQAPGKGLEWVSSISSGSGTIYYADSVKGRFTISRDNPKNSLYLQMNSLRAEDTAVYYCARAYYGNGFSFWGQGTLVTVSS

SEQ ID NO: 61 - protein, 113 aa, Artificial Sequence
DIVMTQSPDSLAVSLGERATINCKSSQSLLNSGNQKNYLTWYQQKPGQPPKLLIYWASTRESGVPDRFSGSGSGTDFTLTISSLQAEDVAVYYCQNVYSYPLTFGQGTKLEIK

SEQ ID NO: 62 - protein, 17 aa, Artificial Sequence
  X is substituted as shown in the specification
XISSGSGTIYYADXVKG

SEQ ID NO: 63 - protein, 17 aa, Artificial Sequence
  X is substituted as shown in the specification
WINTYTGESTYADXFXG

SEQ ID NO: 64 - protein, 448 aa, Artificial Sequence
EVQLVESGGGLVQPGGSLRLSCAASGFTLNNFGMHWVRQAPGKGLEWVSSISSGSGTIYYADSVKGRFTISRDNPKNSLYLQMNSLRAEDTAVYYCARAYYGNGFSFWGQGTLVTVSSASTKGPSVFPLAPSSKSTSGGTAALGCLVKDYFPEPVTVSWNSGALTSGVHTFPAVLQSSGLYSLSSVVTVPSSSLGTQTYICNVNHKPSNTKVDKKVEPKSCDKTHTCPPCPAPELLGGPSVFLFPPKPKDTLMISRTPEVTCVVVDVSHEDPEVKFNWYVDGVEVHNAKTKPREEQYNSTYRVVSVLTVLHQDWLNGKEYKCKVSNKALPAPIEKTISKAKGQPREPQVYTLPPSRDELTKNQVSLTCLVKGFYPSDIAVEWESNGQPENNYKTTPPVLDSDGSFFLYSKLTVDKSRWQQGNVFSCSVMHEALHNHYTQKSLSLSPGK

SEQ ID NO: 65 - protein, 220 aa, Artificial Sequence
DIVMTQSPDSLAVSLGERATINCKSSQSLLNSGNQKNYLTWYQQKPGQPPKLLIYWASTRESGVPDRFSGSGSGTDFTLTISSLQAEDVAVYYCQNVYSYPLTFGQGTKLEIKRTVAAPSVFIFPPSDEQLKSGTASVVCLLNNFYPREAKVQWKVDNALQSGNSQESVTEQDSKDSTYSLSSTLTLSKADYEKHKVYACEVTHQGLSSPVTKSFNRGEC

SEQ ID NO: 66 - DNA, 1347 bp, Artificial Sequence
gaggtgcagctggtggagagcggcggcggcctggtgcagcccggcggcagcctgagactgagctgcgccgccagcggcttcaccctgaacaacttcggcatgcactgggtgagacaggcccccggcaagggcctggagtgggtgagctccatcagcagcggcagcggcaccatctactacgccgacagcgtgaagggcagattcaccatcagcagagacaaccccaagaacagcctgtacctgcagatgaacagcctgagagccgaggacaccgccgtgtactactgcgccagagcctactacggcaacggcttcagcttctggggccagggcaccctggtgaccgtgagcagcgctagcaccaagggcccatccgtcttccccctggcaccctcctccaagagcacctctgggggcacagcggccctgggctgcctggtcaaggactacttccccgaaccggtgacggtgtcgtggaactcaggcgccctgaccagcggcgtgcacaccttcccggctgtcctacagtcctcaggactctactccctcagcagcgtggtgaccgtgccctccagcagcttgggcacccagacctacatctgcaacgtgaatcacaagcccagcaacaccaaggtggacaagaaagttgagcccaaatcttgtgacaaaactcacacatgcccaccgtgcccagcacctgaactcctggggggaccgtcagtcttcctcttccccccaaaacccaaggacaccctcatgatctcccggacccctgaggtcacatgcgtggtggtggacgtgagccacgaagaccctgaggtcaagttcaactggtacgtggacggcgtggaggtgcataatgccaagacaaagccgcgggaggagcagtacaacagcacgtaccgtgtggtcagcgtcctcaccgtcctgcaccaggactggctgaatggcaaggagtacaagtgcaaggtctccaacaaagccctcccagcccccatcgagaaaaccatctccaaagccaaagggcagccccgagaaccacaggtgtacaccctgcccccatcccgggacgagctgaccaagaaccaggtcagcctgacctgcctggtcaaaggcttctatcccagcgacatcgccgtggagtgggagagcaatgggcagccggagaacaactacaagaccacgcctcccgtgctggactccgacggctccttcttcctctatagcaagctcaccgtggacaagagcaggtggcagcaggggaacgtcttctcatgctccgtgatgcatgaggctctgcacaaccactacacgcagaagtccctctccctgtctccgggtaaatga

SEQ ID NO: 67 - DNA, 663 bp, Artificial Sequence
gacatcgtgatgacccagagccccgacagcctggccgtgagcctgggcgagagagccaccatcaactgcaagagcagccagagcctgctgaacagcggcaaccagaagaactacctgacctggtaccagcagaagcccggccagccccccaagctgctgatctactgggccagcaccagagagagcggcgtgcccgacagattcagcggcagcggcagcggcaccgacttcaccctgaccatcagcagcctgcaggccgaggacgtggccgtgtactactgccagaacgtgtacagctaccccctgaccttcggccagggcaccaagctggagatcaagcgaactgtggctgcaccatctgtcttcatcttcccgccatctgatgagcagttgaaatctggaactgcctctgttgtgtgcctgctgaataacttctatcccagagaggccaaagtacagtggaaggtggataacgccctccaatcgggtaactcccaggagagtgtcacagagcaggacagcaaggacagcacctacagcctcagcagcaccctgacgctgagcaaagcagactacgagaaacacaaagtctacgcctgcgaagtcacccatcagggcctgagctcgcccgtcacaaagagcttcaacaggggagagtgttag

SEQ ID NO: 68 - protein, 448 aa, Artificial Sequence
QIQLVQSGSELKKPGESVKVSCKASGYTFTNYGMNWVRQAPGQGLEWMGWINTYTGESTYADGFTGRFVFSSDTSARTAYLQISSLKAEDTAVYFCATLGYGNSLAYWGQGTLVTVSSASTKGPSVFPLAPSSKSTSGGTAALGCLVKDYFPEPVTVSWNSGALTSGVHTFPAVLQSSGLYSLSSVVTVPSSSLGTQTYICNVNHKPSNTKVDKKVEPKSCDKTHTCPPCPAPELLGGPSVFLFPPKPKDTLMISRTPEVTCVVVDVSHEDPEVKFNWYVDGVEVHNAKTKPREEQYNSTYRVVSVLTVLHQDWLNGKEYKCKVSNKALPAPIEKTISKAKGQPREPQVYTLPPSRDELTKNQVSLTCLVKGFYPSDIAVEWESNGQPENNYKTTPPVLDSDGSFFLYSKLTVDKSRWQQGNVFSCSVMHEALHNHYTQKSLSLSPGK

SEQ ID NO: 69 - protein, 220 aa, Artificial Sequence
DIVMTQSPDSLAVSLGERATINCKSSQSLLNSGNQRNYLTWYQQKPGQPPKLLIYWASTRESGVPDRFSGSGSGTDFTLTISSLQAEDVAVYYCQNNYFYPFTFGQGTKLEIKRTVAAPSVFIFPPSDEQLKSGTASVVCLLNNFYPREAKVQWKVDNALQSGNSQESVTEQDSKDSTYSLSSTLTLSKADYEKHKVYACEVTHQGLSSPVTKSFNRGEC

SEQ ID NO: 70 - DNA, 1347 bp, Artificial Sequence
cagatccagctggtgcagagcggcagcgagctgaagaagcccggcgagagcgtgaaggtgagctgcaaggccagcggctacaccttcaccaactacggcatgaactgggtgagacaggcccccggccagggcctggagtggatgggctggatcaacacctacaccggcgagagcacctacgccgacggcttcaccggcagattcgtgttcagcagcgacaccagcgccagaaccgcctacctgcagatcagcagcctgaaggccgaggacaccgccgtgtacttctgcgccaccctgggctacggcaacagcctggcctactggggccagggcaccctggtgaccgtgagcagcgctagcaccaagggcccatccgtcttccccctggcaccctcctccaagagcacctctgggggcacagcggccctgggctgcctggtcaaggactacttccccgaaccggtgacggtgtcgtggaactcaggcgccctgaccagcggcgtgcacaccttcccggctgtcctacagtcctcaggactctactccctcagcagcgtggtgaccgtgccctccagcagcttgggcacccagacctacatctgcaacgtgaatcacaagcccagcaacaccaaggtggacaagaaagttgagcccaaatcttgtgacaaaactcacacatgcccaccgtgcccagcacctgaactcctggggggaccgtcagtcttcctcttccccccaaaacccaaggacaccctcatgatctcccggacccctgaggtcacatgcgtggtggtggacgtgagccacgaagaccctgaggtcaagttcaactggtacgtggacggcgtggaggtgcataatgccaagacaaagccgcgggaggagcagtacaacagcacgtaccgtgtggtcagcgtcctcaccgtcctgcaccaggactggctgaatggcaaggagtacaagtgcaaggtctccaacaaagccctcccagcccccatcgagaaaaccatctccaaagccaaagggcagccccgagaaccacaggtgtacaccctgcccccatcccgggacgagctgaccaagaaccaggtcagcctgacctgcctggtcaaaggcttctatcccagcgacatcgccgtggagtgggagagcaatgggcagccggagaacaactacaagaccacgcctcccgtgctggactccgacggctccttcttcctctatagcaagctcaccgtggacaagagcaggtggcagcaggggaacgtcttctcatgctccgtgatgcatgaggctctgcacaaccactacacgcagaagtccctctccctgtctccgggtaaatga

SEQ ID NO: 71 - DNA, 663 bp, Artificial Sequence
gacatcgtgatgacccagagccccgacagcctggccgtgagcctgggcgagagagccaccatcaactgcaagagcagccagagcctgctgaacagcggcaaccagagaaactacctgacctggtaccagcagaagcccggccagccccccaagctgctgatctactgggccagcaccagagagagcggcgtgcccgacagattcagcggcagcggcagcggcaccgacttcaccctgaccatcagcagcctgcaggccgaggacgtggccgtgtactactgccagaacaactacttctaccccttcaccttcggccagggcaccaagctggagatcaagcgaactgtggctgcaccatctgtcttcatcttcccgccatctgatgagcagttgaaatctggaactgcctctgttgtgtgcctgctgaataacttctatcccagagaggccaaagtacagtggaaggtggataacgccctccaatcgggtaactcccaggagagtgtcacagagcaggacagcaaggacagcacctacagcctcagcagcaccctgacgctgagcaaagcagactacgagaaacacaaagtctacgcctgcgaagtcacccatcagggcctgagctcgcccgtcacaaagagcttcaacaggggagagtgttag

SEQ ID NO: 72 - protein, 17 aa, Artificial Sequence
YISSGSGTIYYADSVKG

SEQ ID NO: 73 - protein, 9 aa, Artificial Sequence
AYYGNAFSF

SEQ ID NO: 74 - protein, 17 aa, Artificial Sequence
TISGGDSYTYYPDSVKG

SEQ ID NO: 75 - protein, 9 aa, Artificial Sequence
SYNANSLPY

SEQ ID NO: 76 - protein, 118 aa, Artificial Sequence
EVQLVESGGGLVQPGGSLRLSCAASGFTLNNFGMHWVRQAPGKGLEWVSYISSGSGTIYYADSVKGRFTISRDNPKNSLYLQMNSLRAEDTAVYYCARAYYGNAFSFWGQGTLVTVSS

SEQ ID NO: 77 - protein, 113 aa, Artificial Sequence
DIVMTQSPSSLAVSLGERATINCKSSQSLLNSGNQKNYLTWYQQKPGQPPKLLIYWASTRESGVPDRFSGSGSGTDFTLTISSLQAEDVAVYYCQNVYSYPLTFGQGTKLEIK

SEQ ID NO: 78 - protein, 118 aa, Artificial Sequence
EVQLVESGGGLVQPGGSLRLSCAASGFTLNNFGMHWVRQAPGKGLEWVSYISSGSGTIYYADSVKGRFTISRDNPKNSLYLQMNSLRAEDTAVYYCARAYYGNGFSFWGQGTLVTVSS

SEQ ID NO: 79 - protein, 118 aa, Artificial Sequence
QIQLVQSGSELKKPGASVKVSCKASGYTFTNYGMNWVRQAPGQGLEWMGWINTYTGESTYADGFTGRFVFSSDTSARTAYLQISSLKAEDTAVYFCATLGYGNSLAYWGQGTLVTVSS

SEQ ID NO: 80 - protein, 113 aa, Artificial Sequence
DIVMTQSPDSLAVTTGERATINCKSSQSLLNSGNQRNYLTWYQQKPGQPPKLLIYWASTRESGVPDRFSGSGSGTDFTLTISSLQAEDVAVYYCQNNYFYPFTFGQGTKLEIK

SEQ ID NO: 81 - protein, 113 aa, Artificial Sequence
DIVMTQSPDFLAVSLGERATINCKSSQSLLNSGNQKNYLTWYQQKPGQPPKLLIYWASTRDSGVPDRFSGSGSGTDFTLTISSLQAEDVAVYYCQNAYFYPFTFGPGTKVDIK

SEQ ID NO: 82 - protein, 118 aa, Artificial Sequence
EVQLVESGGGLVKPGGSLRLSCAASGFTFSSYGMSWVRQAPGKGLEWVSTISGGDSYTYYPDSVKGRFTISRDIAKNSLYLQMNSLRAEDTAVYYCARSYNANSLPYWGQGTLVTVSS

SEQ ID NO: 83 - protein, 118 aa, Artificial Sequence
EVQLVESGGGLVKPGGSLRLSCAASGFTFSSYGMSWVRQAPGKGLEWVSTISGGDSYTYYPDSVKGRFTISRDNAKNSLYLQMNSLRAEDTAVYYCARSYNGNSLPYWGQGTLVTVSS

SEQ ID NO: 84 - protein, 448 aa, Artificial Sequence
EVQLVESGGGLVQPGGSLRLSCAASGFTLNNFGMHWVRQAPGKGLEWVSYISSGSGTIYYADSVKGRFTISRDNPKNSLYLQMNSLRAEDTAVYYCARAYYGNAFSFWGQGTLVTVSSASTKGPSVFPLAPSSKSTSGGTAALGCLVKDYFPEPVTVSWNSGALTSGVHTFPAVLQSSGLYSLSSVVTVPSSSLGTQTYICNVNHKPSNTKVDKKVEPKSCDKTHTCPPCPAPELLGGPSVFLFPPKPKDTLMISRTPEVTCVVVDVSHEDPEVKFNWYVDGVEVHNAKTKPREEQYNSTYRVVSVLTVLHQDWLNGKEYKCKVSNKALPAPIEKTISKAKGQPREPQVYTLPPSRDELTKNQVSLTCLVKGFYPSDIAVEWESNGQPENNYKTTPPVLDSDGSFFLYSKLTVDKSRWQQGNVFSCSVMHEALHNHYTQKSLSLSPGK

SEQ ID NO: 85 - protein, 220 aa, Artificial Sequence; identical to SEQ ID NO: 65

SEQ ID NO: 86 - protein, 448 aa, Artificial Sequence; identical to SEQ ID NO: 84

SEQ ID NO: 87 - protein, 220 aa, Artificial Sequence
DIVMTQSPSSLAVSLGERATINCKSSQSLLNSGNQKNYLTWYQQKPGQPPKLLIYWASTRESGVPDRFSGSGSGTDFTLTISSLQAEDVAVYYCQNVYSYPLTFGQGTKLEIKRTVAAPSVFIFPPSDEQLKSGTASVVCLLNNFYPREAKVQWKVDNALQSGNSQESVTEQDSKDSTYSLSSTLTLSKADYEKHKVYACEVTHQGLSSPVTKSFNRGEC

SEQ ID NO: 88 - protein, 448 aa, Artificial Sequence
EVQLVESGGGLVQPGGSLRLSCAASGFTLNNFGMHWVRQAPGKGLEWVSYISSGSGTIYYADSVKGRFTISRDNPKNSLYLQMNSLRAEDTAVYYCARAYYGNGFSFWGQGTLVTVSSASTKGPSVFPLAPSSKSTSGGTAALGCLVKDYFPEPVTVSWNSGALTSGVHTFPAVLQSSGLYSLSSVVTVPSSSLGTQTYICNVNHKPSNTKVDKKVEPKSCDKTHTCPPCPAPELLGGPSVFLFPPKPKDTLMISRTPEVTCVVVDVSHEDPEVKFNWYVDGVEVHNAKTKPREEQYNSTYRVVSVLTVLHQDWLNGKEYKCKVSNKALPAPIEKTISKAKGQPREPQVYTLPPSRDELTKNQVSLTCLVKGFYPSDIAVEWESNGQPENNYKTTPPVLDSDGSFFLYSKLTVDKSRWQQGNVFSCSVMHEALHNHYTQKSLSLSPGK

SEQ ID NO: 89 - protein, 220 aa, Artificial Sequence; identical to SEQ ID NO: 65

SEQ ID NO: 90 - protein, 448 aa, Artificial Sequence
QIQLVQSGSELKKPGASVKVSCKASGYTFTNYGMNWVRQAPGQGLEWMGWINTYTGESTYADGFTGRFVFSSDTSARTAYLQISSLKAEDTAVYFCATLGYGNSLAYWGQGTLVTVSSASTKGPSVFPLAPSSKSTSGGTAALGCLVKDYFPEPVTVSWNSGALTSGVHTFPAVLQSSGLYSLSSVVTVPSSSLGTQTYICNVNHKPSNTKVDKKVEPKSCDKTHTCPPCPAPELLGGPSVFLFPPKPKDTLMISRTPEVTCVVVDVSHEDPEVKFNWYVDGVEVHNAKTKPREEQYNSTYRVVSVLTVLHQDWLNGKEYKCKVSNKALPAPIEKTISKAKGQPREPQVYTLPPSRDELTKNQVSLTCLVKGFYPSDIAVEWESNGQPENNYKTTPPVLDSDGSFFLYSKLTVDKSRWQQGNVFSCSVMHEALHNHYTQKSLSLSPGK

SEQ ID NO: 91 - protein, 220 aa, Artificial Sequence
DIVMTQSPDSLAVTTGERATINCKSSQSLLNSGNQRNYLTWYQQKPGQPPKLLIYWASTRESGVPDRFSGSGSGTDFTLTISSLQAEDVAVYYCQNNYFYPFTFGQGTKLEIKRTVAAPSVFIFPPSDEQLKSGTASVVCLLNNFYPREAKVQWKVDNALQSGNSQESVTEQDSKDSTYSLSSTLTLSKADYEKHKVYACEVTHQGLSSPVTKSFNRGEC

SEQ ID NO: 92 - protein, 448 aa, Artificial Sequence
QVQLVQSGSELKKPGESVKVSCKASGYTFTNYGMNWVRQAPGQGLEWMGWINTYTGESTYADGFTGRFVFSMDTSASTAYLQISSLKAEDMAMYFCATLGYGNSLAYWGQGTLVTVSSASTKGPSVFPLAPSSKSTSGGTAALGCLVKDYFPEPVTVSWNSGALTSGVHTFPAVLQSSGLYSLSSVVTVPSSSLGTQTYICNVNHKPSNTKVDKKVEPKSCDKTHTCPPCPAPELLGGPSVFLFPPKPKDTLMISRTPEVTCVVVDVSHEDPEVKFNWYVDGVEVHNAKTKPREEQYNSTYRVVSVLTVLHQDWLNGKEYKCKVSNKALPAPIEKTISKAKGQPREPQVYTLPPSRDELTKNQVSLTCLVKGFYPSDIAVEWESNGQPENNYKTTPPVLDSDGSFFLYSKLTVDKSRWQQGNVFSCSVMHEALHNHYTQKSLSLSPGK

SEQ ID NO: 93 - protein, 220 aa, Artificial Sequence; identical to SEQ ID NO: 69

SEQ ID NO: 94 - protein, 448 aa, Artificial Sequence; identical to SEQ ID NO: 68

SEQ ID NO: 95 - protein, 220 aa, Artificial Sequence
DIVMTQSPDFLAVSLGERATINCKSSQSLLNSGNQKNYLTWYQQKPGQPPKLLIYWASTRDSGVPDRFSGSGSGTDFTLTISSLQAEDVAVYYCQNAYFYPFTFGPGTKVDIKRTVAAPSVFIFPPSDEQLKSGTASVVCLLNNFYPREAKVQWKVDNALQSGNSQESVTEQDSKDSTYSLSSTLTLSKADYEKHKVYACEVTHQGLSSPVTKSFNRGEC

SEQ ID NO: 96 - protein, 448 aa, Artificial Sequence; identical to SEQ ID NO: 92

SEQ ID NO: 97 - protein, 220 aa, Artificial Sequence; identical to SEQ ID NO: 69

SEQ ID NO: 98 - protein, 448 aa, Artificial Sequence
EVQLVESGGGLVKPGGSLRLSCAASGFTFSSYGMSWVRQAPGKGLEWVSTISGGDSYTYYPDSVKGRFTISRDIAKNSLYLQMNSLRAEDTAVYYCARSYNANSLPYWGQGTLVTVSSASTKGPSVFPLAPSSKSTSGGTAALGCLVKDYFPEPVTVSWNSGALTSGVHTFPAVLQSSGLYSLSSVVTVPSSSLGTQTYICNVNHKPSNTKVDKKVEPKSCDKTHTCPPCPAPELLGGPSVFLFPPKPKDTLMISRTPEVTCVVVDVSHEDPEVKFNWYVDGVEVHNAKTKPREEQYNSTYRVVSVLTVLHQDWLNGKEYKCKVSNKALPAPIEKTISKAKGQPREPQVYTLPPSRDELTKNQVSLTCLVKGFYPSDIAVEWESNGQPENNYKTTPPVLDSDGSFFLYSKLTVDKSRWQQGNVFSCSVMHEALHNHYTQKSLSLSPGK

SEQ ID NO: 99 - protein, 220 aa, Artificial Sequence; identical to SEQ ID NO: 69

SEQ ID NO: 100 - protein, 448 aa, Artificial Sequence
EVQLVESGGGLVKPGGSLRLSCAASGFTFSSYGMSWVRQAPGKGLEWVSTISGGDSYTYYPDSVKGRFTISRDNAKNSLYLQMNSLRAEDTAVYYCARSYNGNSLPYWGQGTLVTVSSASTKGPSVFPLAPSSKSTSGGTAALGCLVKDYFPEPVTVSWNSGALTSGVHTFPAVLQSSGLYSLSSVVTVPSSSLGTQTYICNVNHKPSNTKVDKKVEPKSCDKTHTCPPCPAPELLGGPSVFLFPPKPKDTLMISRTPEVTCVVVDVSHEDPEVKFNWYVDGVEVHNAKTKPREEQYNSTYRVVSVLTVLHQDWLNGKEYKCKVSNKALPAPIEKTISKAKGQPREPQVYTLPPSRDELTKNQVSLTCLVKGFYPSDIAVEWESNGQPENNYKTTPPVLDSDGSFFLYSKLTVDKSRWQQGNVFSCSVMHEALHNHYTQKSLSLSPGK

SEQ ID NO: 101 - protein, 220 aa, Artificial Sequence; identical to SEQ ID NO: 69